European Patent Application EP 4 560 017 A1, published May 28, 2025. Title: Plant biomass saccharifying enzyme composition. Applicant: KAO CORPORATION. The sequence listing filed with the application follows.

SEQUENCE LISTING (49 sequences)

SEQ ID NO: 1 - DNA, 1089 bp, Aspergillus niger
  source 1..1089: mol_type = genomic DNA
  CDS 1..1089
atgcatttcctccagaacgccgttgtggccgccactatgggcgctgcgctggccgccgctgctcctctcgagaagcgctcctgcactttcacctccgcctctgctgccaagtccggcaagtcctcttgctccaccatcaccctcgacaacatcgcggtccccgctggtgagactcttgacttgactggcctcaagaagggtaccaccgtcatcttcgagggtgagaccaccttcggctacaaggaatggaagggtcccctgatctccatgtccggtaccgacatcaccgtcaagcaggcctccggtgccaagatcaactgcgacggtgctcgctggtgggacggcaagggtagcaacggtggcaagaccaagcccaagttcttccaggcccacaagctcgaccagtccagcatcaccggcctgaaggtctacaacacccctgtccagggtttcagcattctggccgaccacctgaccatcaccgatgtgaccatcgacaactccgccggtaccagcaagggtcacaacaccgatgcctttgacattggccagagtacctacatcaccattgacggtgccaccgtctacaaccaggatgactgcctggccatcaactcgggtgagcacatcaccttcaccaacggctactgtgatggtggccacggtctctccatcggttccatcggtggccgcagtgacaacaccgtcaacgacgtgaccatctccaactccaaggtgctcaactcccagaacggtgtccgcatcaagaccatctacggcaagactggcactgtcgagaacgtcaagtttgaggacatcaccctgtccgacatcagcaagtacggtattgtcgttgagcaggactacgagaacggcagccccaccggcacgcccaccaacggtgtcaaggttgaggacatcactttcaagaaggtcaccggcagcgtcaagagctctggtactgacatctacatcctgtgcggttccggcagctgctcgaactggacctggagcggtgttgatgtgactggcggcaagaagagcagcaagtgcaagaacgtcccctcgggcgcttcctgcagcgattaa

SEQ ID NO: 2 - protein, 362 aa, Aspergillus niger
MHFLQNAVVAATMGAALAAAAPLEKRSCTFTSASAAKSGKSSCSTITLDNIAVPAGETLDLTGLKKGTTVIFEGETTFGYKEWKGPLISMSGTDITVKQASGAKINCDGARWWDGKGSNGGKTKPKFFQAHKLDQSSITGLKVYNTPVQGFSILADHLTITDVTIDNSAGTSKGHNTDAFDIGQSTYITIDGATVYNQDDCLAINSGEHITFTNGYCDGGHGLSIGSIGGRSDNTVNDVTISNSKVLNSQNGVRIKTIYGKTGTVENVKFEDITLSDISKYGIVVEQDYENGSPTGTPTNGVKVEDITFKKVTGSVKSSGTDIYILCGSGSCSNWTWSGVDVTGGKKSSKCKNVPSGASCSD

SEQ ID NO: 3 - DNA, 1107 bp, Aspergillus niger
  source 1..1107: mol_type = genomic DNA
  CDS 1..1107
atgcactcttaccagcttcttggcctggccgctgtcggctccctcgtctctgccgcccccgctccttctcgcgtctccgagttcgctaagaaggcctctacctgcaccttcacctctgcctctgaggccagcgagagcatctccagctgctccgatgttgtcctgagcagcatcgaggtccccgctggcgagaccctggacctgtccgatgctgctgatggctccaccatcaccttcgagggcaccacttccttcggatacaaggaatggaagggtcccctgatccgcttcggtggtaaggatctgaccgtcaccatggccgacggcgctgtcatcgacggtgacggttcccgctggtgggacagcaagggtaccaacggtggcaagaccaagcccaagttcatgtacatccacgacgttgaggactcgaccttcaagggcatcaacatcaagaatactcccgtccaggccatcagtgtccaggctaccaacgtccacctgaacgacttcaccatcgacaactccgacggtgatgacaacggtggccacaacaccgacggtttcgacatcagcgagtccaccggtgtctacatcagcggtgctaccgtcaagaaccaggacgactgcattgccatcaactctggcgagagcatctctttcaccggcggtacctgctccggtggccacggtctctccatcggctctgtcggtggccgtgatgacaacaccgtcaagaacgtgaccatctccgactccactgtcagcaactccgccaatggtgtccgcatcaagaccatctacaaggagaccggcgatgtcagcgagatcacctactccaacatccagctctccggcatcaccgactacggtatcgtcatcgagcaggactacgagaacggctctcccaccggcaccccctccaccggtatccccatcactgatgtcactgttgacggtgtcaccggcactcttgaggatgacgccacccaggtctacattctctgcggtgacggctcttgctctgactggacctggtccggtgttgacctctctggtggcaagaccagcgataaatgcgagaacgttccttccggtgcttcttgctaa

SEQ ID NO: 4 - protein, 368 aa, Aspergillus niger
MHSYQLLGLAAVGSLVSAAPAPSRVSEFAKKASTCTFTSASEASESISSCSDVVLSSIEVPAGETLDLSDAADGSTITFEGTTSFGYKEWKGPLIRFGGKDLTVTMADGAVIDGDGSRWWDSKGTNGGKTKPKFMYIHDVEDSTFKGINIKNTPVQAISVQATNVHLNDFTIDNSDGDDNGGHNTDGFDISESTGVYISGATVKNQDDCIAINSGESISFTGGTCSGGHGLSIGSVGGRDDNTVKNVTISDSTVSNSANGVRIKTIYKETGDVSEITYSNIQLSGITDYGIVIEQDYENGSPTGTPSTGIPITDVTVDGVTGTLEDDATQVYILCGDGSCSDWTWSGVDLSGGKTSDKCENVPSGASC

SEQ ID NO: 5 - DNA, 1089 bp, Aspergillus niger
  source 1..1089: mol_type = genomic DNA
  CDS 1..1089
atgcactcgtttgcttctcttctcgcctacggcctggtcgccggcgccaccttcgcttctgcctctcctatcgaagctcgagacagctgcacgttcaccaccgctgccgctgctaaagcgggcaaggcgaaatgctctactatcacccttaacaacatcgaagttccagctggaaccaccctcgacctgaccggtctcaccagcggtaccaaggtcatcttcgagggcaccacgaccttccagtacgaagaatgggcaggccccttgatctccatgagtggcgaacatatcaccgtcactggtgcctccggccacctcatcaattgcgatggtgcgcgctggtgggatggcaagggaaccagcggaaagaagaagcccaagttcttttacgcccatggccttgactcctcgtctattactggattaaacatcaaaaacactccccttatggcgtttagtgtccaggcgaatgacattacgtttaccgatgttaccatcaataatgcggatggcgacacccagggtggacacaacactgatgcgttcgatgttggtaactcggtcggggtgaatatcattaagccttgggtccataaccaggatgactgtcttgcgattaactctggcgagaacatctggttcaccggcggcacctgcattggcggccacggtctctccatcggctctgtcggcgaccgctccaacaacgtcgtcaagaacgtcaccatcgaacactccaccgtgagcaattccgaaaacgccgtccgaatcaagaccatctctggcgccactggctccgtgtctgagattacatactccaacatcgtcatgtccggcatctccgattacggcgtggtcattcagcaggattacgaagacggcaagcctacgggtaagccgacgaacggtgtcactattcaggatgtcaagctggagagcgtgaccggtagcgtggatagtaaggctactgagatctatcttctttgcgggtctggtagctgctcggactggacctgggacgatgtgaaggttactggggggaagaagtccaccgcttgcaagaacttcccttcggtggcctcttgctag

SEQ ID NO: 6 - protein, 362 aa, Aspergillus niger
MHSFASLLAYGLVAGATFASASPIEARDSCTFTTAAAAKAGKAKCSTITLNNIEVPAGTTLDLTGLTSGTKVIFEGTTTFQYEEWAGPLISMSGEHITVTGASGHLINCDGARWWDGKGTSGKKKPKFFYAHGLDSSSITGLNIKNTPLMAFSVQANDITFTDVTINNADGDTQGGHNTDAFDVGNSVGVNIIKPWVHNQDDCLAINSGENIWFTGGTCIGGHGLSIGSVGDRSNNVVKNVTIEHSTVSNSENAVRIKTISGATGSVSEITYSNIVMSGISDYGVVIQQDYEDGKPTGKPTNGVTIQDVKLESVTGSVDSKATEIYLLCGSGSCSDWTWDDVKVTGGKKSTACKNFPSVASC

SEQ ID NO: 7 - DNA, 1122 bp, Aspergillus niger
  source 1..1122: mol_type = genomic DNA
  CDS 1..1122
atgaagtacgctgctgctctcacggctgttgccgccctcgctgcccgcgccgctgctgtcggtgtctccggcactcccgtgggtttcgcctcctccgccactggtggtggtgatgctacccccgtctaccctaccaccaccgatgagctggtctcttacctcggtgatgacgaggcccgtgtcattgtcctgtccaagactttcgacttcactgacactgagggcactaccacgaccaccggttgcgctccctggggtactgcctccggctgccagctggccatcaacaaggacgactggtgcaccaactacgagcccgatgctcccaccaccaccgtcacctacaacactgctggtgaactcggtatcaccgtcaactccaacaagtccttgatcggtgagggtaccagcggtgtcatcaagggccgtggtctccgcatggtcagcggtgtctccaacatcatcatccagaacattgctgtcaccgacatcaaccccgagtacgtctggggtggtgacgccatcaccctcgacgaggctgacttggtctggattgaccacgttaccactgcccgcattggtcgccagcactacgtcctcggtaccgacgccgacagccgtgtctccatcaccaacaactacatcaacggcgagtctgactactctgctacttgcgacggccaccactactggaacgtgtaccttgacggctctagcgacaaggtcaccttcagtggcaactacctgtacaagacctccggccgtgcccccaaggtccaggacaacacctacctccacatctacaacaactactgggagaacaactcgggccacgctttcgagatcggctccggtggctacgtcctcgccgagggtaactacttctccaacgtcgacaccgtcctcgagaccgacaccttcgagggtgctctcttctcctctgacagcgcctcctccacctgcgagtcctacattggccgttcctgcgttgccaacgtcaacggcggtgacctcaccggcacctccaccaccgtcctctccaacctcagcggcgacaccctcccctctgctgatgctgccagcaccagccccgcctccaacgctggtcagggtaacctgtaa

SEQ ID NO: 8 - protein, 373 aa, Aspergillus niger
MKYAAALTAVAALAARAAAVGVSGTPVGFASSATGGGDATPVYPTTTDELVSYLGDDEARVIVLSKTFDFTDTEGTTTTTGCAPWGTASGCQLAINKDDWCTNYEPDAPTTTVTYNTAGELGITVNSNKSLIGEGTSGVIKGRGLRMVSGVSNIIIQNIAVTDINPEYVWGGDAITLDEADLVWIDHVTTARIGRQHYVLGTDADSRVSITNNYINGESDYSATCDGHHYWNVYLDGSSDKVTFSGNYLYKTSGRAPKVQDNTYLHIYNNYWENNSGHAFEIGSGGYVLAEGNYFSNVDTVLETDTFEGALFSSDSASSTCESYIGRSCVANVNGGDLTGTSTTVLSNLSGDTLPSADAASTSPASNAGQGNL

SEQ ID NO: 9 - DNA, 1140 bp, Aspergillus niger
  source 1..1140: mol_type = genomic DNA
  CDS 1..1140
atgaagtactctactatcttcagcgctgctgccgctgttttcgctggttccgccgctgcagtcggcgtgtccggctctgctgagggtttcgccgagggcgtcaccggtggcggtgatgccacccccgtctaccccgacactatcgatgagctggtctcttaccttggagacgatgaggcccgcgtcattgtcctgaccaagaccttcgacttcaccgacagcgaaggtaccaccactggcactggttgcgctccctggggtaccgcttccgcctgccaggttgctattgaccaggacgactggtgcgagaactacgagcccgatgctccctctatcagcgttgaatactacaacgctggtgtcctcggtatcaccgtcacctccaacaagtccctcatcggtgagggctcctctggtgcaatcaagggcaagggtctccgtattgtcagcggtgctgagaacatcatcatccagaacatcgcggttaccgacatcaaccccaagtacgtctggggtggtgatgctattactcttgatgactgcgacctggtctggatcgaccatgttactaccgcccgcatcggtcgccagcactacgtccttggaaccagcgccgacaaccgcgtctctctcaccaacaactacattgacggtgtctccgactactccgccacctgcgatggctaccactactggggcatctacctcgatggtgacgccgacttggtcaccatgaagggcaactacatctaccacacctccggccgtagccccaaggtccaggacaacactctcctccactgtgtcaacaactacttctacgacatctccggccacgcttttgagatcggtgagggtggctacgtcctggctgagggcaacgttttccagaacgtcgacaccgtccttgagacctacgagggcgcggccttcaccgtcccctccaccaccgccggtgaagtctgctccacctaccttggccgtgactgtgtcatcaacggcttcggctcctccggcactttctccgaggacagcacctctttcctctccgacttcgagggcaagaacattgcctctgcttccgcttacacctctgttgcctctagcgttgttgctaacgccggtcagggcaacctgtaa

SEQ ID NO: 10 - protein, 379 aa, Aspergillus niger
MKYSTIFSAAAAVFAGSAAAVGVSGSAEGFAEGVTGGGDATPVYPDTIDELVSYLGDDEARVIVLTKTFDFTDSEGTTTGTGCAPWGTASACQVAIDQDDWCENYEPDAPSISVEYYNAGVLGITVTSNKSLIGEGSSGAIKGKGLRIVSGAENIIIQNIAVTDINPKYVWGGDAITLDDCDLVWIDHVTTARIGRQHYVLGTSADNRVSLTNNYIDGVSDYSATCDGYHYWGIYLDGDADLVTMKGNYIYHTSGRSPKVQDNTLLHCVNNYFYDISGHAFEIGEGGYVLAEGNVFQNVDTVLETYEGAAFTVPSTTAGEVCSTYLGRDCVINGFGSSGTFSEDSTSFLSDFEGKNIASASAYTSVASSVVANAGQGNL

SEQ ID NO: 11 - DNA, 1887 bp, Aspergillus niger
  source 1..1887: mol_type = genomic DNA
  CDS 1..1884
atggtggccttttcagctctttcgggcgtcagcgccgtttctttactactatccctcgttcaaaatgcacacggaatctccttgaaggtctccacccagggtggcaactcatccagccccatcctatatggcttcatgtttgaggatatcaatcactcaggagatggaggaatttatgggcaaatgctgcagaaccctggccttcagggaacggcgcctaatctgactgcctgggcggctgtcggtgacgctaccatcgccattgatggcgacagtccattgacctctgccatccccagcaccatcaagcttaatattgcggacgatgctaccggtgcggtgggtctcaccaatgagggatattggggcatcccagtcgatggcagcgaattccatagttccttctggataaagggagattactccggcgacatcaccgtccgactggttggaaactacaccggcacggagtacggctctaccactatcacccatacgtccacagcagacaactttacccaagcctccgtcaagttccccaccaccaaggctccagatggcaacgttttgtacgagctcacagttgatggaagcgtggctgctggctcgtctttgaacttcggctacttgacgctttttggcgaaacctataagtcaagggaaaatggcctgaagccccagcttgccaatgtgttggatgatatgaaaggatccttcctgagatttcccggcggtaacaaccttgagggaaacagcgcagaaaaccgctggaagtggaacgagacaatcggcgatctttgggatcgtcccggacgtgaaggcacttggacttactataacaccgacggactgggccttcacgaatacttttactggtgtgaggatttggggctcgtaccggtgctcggtgtctgggatgggttcgctctggagtcgggtggcaacacccccctcacgggcgacgcactgaccccttatatcgacgatgtcttgaacgagctcgagtacatcttgggtgatacgagcacgacctatggagcgtggcgcgcggcaaacggacaggaggagccgtggaaccttaccatggtcgagattggcaatgaggacatgctgggaggcggatgcgagtcctacgcggaacgtttcactgccttctatgatgcgattcatgctgcttatccggaccttatcctgattgccagcaccagcgaggcggattgcttgcccgagtcaatgcccgagggtagctgggtcgactaccacgactacagcacgcctgatggactggtgggccagttcaactacttcgacaatttaaaccgctcggtaccatacttcatcggcgagtactcgcgctgggagattgactggcccaacatgaagggatcggtcgctgaagccgtcttcatgatcgggttcgagaggaacagcgacgtggtgaagatggcggcgtatgcgcctttgctccagctaatcaactcgactcagtggacgccggacctgatcggatacacgcagtcacccggtgacattttcctgtcgaccagctactacgtgcaggagatgttctcgcgcaaccggggtgatacaattaaggaggtgacgtcggacagcgacttcggaccgttgtactgggttgcgtcgagcgccggggactcgtactacatgaagctggccaactatggctccgagacgcaagacctcacggtgagcatcccaggaacgagcacaggcaagttgacggtgctggcggacagtgatccggatgcgtataactcggacacccagacgctggtcacgccgagtgaatcgacggtgcaggcgagcaatggcacttttacctttagtttgccggcatgggcggtggctgtcctggcggcgaactag

SEQ ID NO: 12 - protein, 628 aa, Aspergillus niger
MVAFSALSGVSAVSLLLSLVQNAHGISLKVSTQGGNSSSPILYGFMFEDINHSGDGGIYGQMLQNPGLQGTAPNLTAWAAVGDATIAIDGDSPLTSAIPSTIKLNIADDATGAVGLTNEGYWGIPVDGSEFHSSFWIKGDYSGDITVRLVGNYTGTEYGSTTITHTSTADNFTQASVKFPTTKAPDGNVLYELTVDGSVAAGSSLNFGYLTLFGETYKSRENGLKPQLANVLDDMKGSFLRFPGGNNLEGNSAENRWKWNETIGDLWDRPGREGTWTYYNTDGLGLHEYFYWCEDLGLVPVLGVWDGFALESGGNTPLTGDALTPYIDDVLNELEYILGDTSTTYGAWRAANGQEEPWNLTMVEIGNEDMLGGGCESYAERFTAFYDAIHAAYPDLILIASTSEADCLPESMPEGSWVDYHDYSTPDGLVGQFNYFDNLNRSVPYFIGEYSRWEIDWPNMKGSVAEAVFMIGFERNSDVVKMAAYAPLLQLINSTQWTPDLIGYTQSPGDIFLSTSYYVQEMFSRNRGDTIKEVTSDSDFGPLYWVASSAGDSYYMKLANYGSETQDLTVSIPGTSTGKLTVLADSDPDAYNSDTQTLVTPSESTVQASNGTFTFSLPAWAVAVLAAN

SEQ ID NO: 13 - DNA, 1053 bp, Aspergillus niger
  source 1..1053: mol_type = genomic DNA
  CDS 1..1050
atgatctactctctgcttctctctgcattgcctctgctcagcagcgccgccctgacctaccgcggggcggatatctcctcccttttgatcgaggaagatgccggcatcagctataagaatttgaatggcgagacccaggcattggaggatattctggtcaacaatggcgtcaactcgatccgacagagggtgtgggtagaccccagcgatggctcgtacgatctcgactataatctcaagctggccaagcgtgttcaggccgcgggtatgagcatttacttggatctgcatctcagtgatacgtgggcagatcccagtgatcagactacccctaccggttggtcgaccacggacatcgacacactcacctggcaactgtataactacacgctcgacgtctgcaacactttcgcagagaatgacattgacatagagattgtctccattggtaatgagatcagcagcggacttctctggccattgggcaaaaccagcaactatgacaatatcgcgaagctgctgcactccggcgcctggggagtgaaggactccaaccaggccacaaccccgaagattatgatccacctggacaatggatgggactgggaggaacaagaatacttctacaagactgtcctggccacggggtcgctgctctccacggatttcgacctcatgggagtctcgtactatccattctacagctcggaagctaccctgtcggcgctccagaccagcctcacgaacatgcaatcgaactacgataagtccgtggtggtggtggagacgaactggcccgtgtcttgcccggacccggagtattcattcccgtcggatctcagctcgatccccttctcggccgcaggacaggaggagttcctcgagaagctcgcagaggtggtagagggcgtcacggacggactgggtatttattactgggaaccggcgtgggtcgacaatgccgcgctaggatccagctgtgcggacaacctgatggtggatattgacacagatgaagtcctggagagtgtcaccgtgtttgaggacctctga

SEQ ID NO: 14 - protein, 350 aa, Aspergillus niger
MIYSLLLSALPLLSSAALTYRGADISSLLIEEDAGISYKNLNGETQALEDILVNNGVNSIRQRVWVDPSDGSYDLDYNLKLAKRVQAAGMSIYLDLHLSDTWADPSDQTTPTGWSTTDIDTLTWQLYNYTLDVCNTFAENDIDIEIVSIGNEISSGLLWPLGKTSNYDNIAKLLHSGAWGVKDSNQATTPKIMIHLDNGWDWEEQEYFYKTVLATGSLLSTDFDLMGVSYYPFYSSEATLSALQTSLTNMQSNYDKSVVVVETNWPVSCPDPEYSFPSDLSSIPFSAAGQEEFLEKLAEVVEGVTDGLGIYYWEPAWVDNAALGSSCADNLMVDIDTDEVLESVTVFEDL

SEQ ID NO: 15 - DNA, 22 bp, synthetic construct
  source 1..22: mol_type = other DNA
taaaggggcggccgctcaagag

SEQ ID NO: 16 - DNA, 20 bp, synthetic construct
  source 1..20: mol_type = other DNA
agcttcggcctctcttttct

SEQ ID NO: 17 - DNA, 35 bp, synthetic construct
  source 1..35: mol_type = other DNA
agagaggccgaagctgctcctctcgagaagcgctc

SEQ ID NO: 18 - DNA, 35 bp, synthetic construct
  source 1..35: mol_type = other DNA
gcggccgcccctttattaatcgctgcaggaagcgc

SEQ ID NO: 19 - DNA, 35 bp, synthetic construct
  source 1..35: mol_type = other DNA
agagaggccgaagctgtcggtgtctccggcactcc

SEQ ID NO: 20 - DNA, 35 bp, synthetic construct
  source 1..35: mol_type = other DNA
gcggccgcccctttattacaggttaccctgaccag

SEQ ID NO: 21 - DNA, 35 bp, synthetic construct
  source 1..35: mol_type = other DNA
agagaggccgaagctatctccttgaaggtctccac

SEQ ID NO: 22 - DNA, 35 bp, synthetic construct
  source 1..35: mol_type = other DNA
gcggccgcccctttactagttcgccgccaggacag

SEQ ID NO: 23 - DNA, 35 bp, synthetic construct
  source 1..35: mol_type = other DNA
agagaggccgaagctgccctgacctaccgcggggc

SEQ ID NO: 24 - DNA, 35 bp, synthetic construct
  source 1..35: mol_type = other DNA
gcggccgcccctttatcagaggtcctcaaacacgg

SEQ ID NO: 25 - DNA, 35 bp, synthetic construct
  source 1..35: mol_type = other DNA
atatctggtggatctatgcattatgcgcaaatgct

SEQ ID NO: 26 - DNA, 35 bp, synthetic construct
  source 1..35: mol_type = other DNA
acaacgagaaaagaaaacacctggaaagcttgccg

SEQ ID NO: 27 - DNA, 23 bp, synthetic construct
  source 1..23: mol_type = other DNA
ttcttttctcgttgtctcactct

SEQ ID NO: 28 - DNA, 22 bp, synthetic construct
  source 1..22: mol_type = other DNA
agatccaccagatatgtcagga

SEQ ID NO: 29 - DNA, 35 bp, synthetic construct
  source 1..35: mol_type = other DNA
taccacggcaaaggtttcttttctcgttgtctcac

SEQ ID NO: 30 - DNA, 35 bp, synthetic construct
  source 1..35: mol_type = other DNA
tcgggcttcgaacaggatggcgtcgctttctaggc

SEQ ID NO: 31 - DNA, 21 bp, synthetic construct
  source 1..21: mol_type = other DNA
ctgttcgaagcccgaatgtag

SEQ ID NO: 32 - DNA, 20 bp, synthetic construct
  source 1..20: mol_type = other DNA
acctttgccgtggtactggg

SEQ ID NO: 33 - DNA, 35 bp, synthetic construct
  source 1..35: mol_type = other DNA
atgcccaccatatctctgttcgaagcccgaatgta

SEQ ID NO: 34 - DNA, 35 bp, synthetic construct
  source 1..35: mol_type = other DNA
tcacgtttccaggttagatccaccagatatgtcag

SEQ ID NO: 35 - DNA, 20 bp, synthetic construct
  source 1..20: mol_type = other DNA
aacctggaaacgtgagatgt

SEQ ID NO: 36 - DNA, 20 bp, synthetic construct
  source 1..20: mol_type = other DNA
agatatggtgggcattgcgt

SEQ ID NO: 37 - DNA, 35 bp, synthetic construct
  source 1..35: mol_type = other DNA
taccacggcaaaggtaacctggaaacgtgagatgt

SEQ ID NO: 38 - DNA, 35 bp, synthetic construct
  source 1..35: mol_type = other DNA
acaacgagaaaagaatcatgaatatatgcttggta

SEQ ID NO: 39 - DNA, 21 bp, synthetic construct
  source 1..21: mol_type = other DNA
atgtatcggaagttggccgtc

SEQ ID NO: 40 - DNA, 20 bp, synthetic construct
  source 1..20: mol_type = other DNA
agatatggtgggcattgcgt

SEQ ID NO: 41 - DNA, 35 bp, synthetic construct
  source 1..35: mol_type = other DNA
atgcccaccatatctcaagtcttcgtactctatcg

SEQ ID NO: 42 - DNA, 35 bp, synthetic construct
  source 1..35: mol_type = other DNA
aacttccgatacatgatgattatttgtgcgtgttt

SEQ ID NO: 43 - DNA, 20 bp, synthetic construct
  source 1..20: mol_type = other DNA
agctccgtggcgaaagcctg

SEQ ID NO: 44 - DNA, 20 bp, synthetic construct
  source 1..20: mol_type = other DNA
gatgattatttgtgcgtgtt

SEQ ID NO: 45 - DNA, 35 bp, synthetic construct
  source 1..35: mol_type = other DNA
gcacaaataatcatcatgatctactctctgcttct

SEQ ID NO: 46 - DNA, 35 bp, synthetic construct
  source 1..35: mol_type = other DNA
tttcgccacggagcttcagaggtcctcaaacacgg

SEQ ID NO: 47 - DNA, 3317 bp, Trichoderma reesei
  source 1..3317: mol_type = genomic DNA
tctgtccattgaggagcgtgatgtctaggcgcatcactaacacggagctgtatgaccggcagctcaacggacttctcttcgttcaacggcagtctatttgcggtacacgaatggatctttcttcctggtcttgaagtgccgcagtggcgtgcgaatgtatagatgtctcgctacctagaaaagctggcttttctgacagggtcccttccacctctcctaccaacgacaaactgaacaagtatctggcggtttcccaacgccgaataggccagtcgccaatactccctccagccctgattgggcccctcgaagtatcgccatgtctgtgtgttgagattattcgatggacgtcactcccccaacctacaggaagagcaaaatgggagcagtgttctgcaatgagctatataatagatcgctcgatctcatacaaattgtatgctcagtcaatacaacgagcggttccaagatcccttctccaacgaccctcgaaacattgcaacccggtgcagcctgaacttgttcgtatagcctagaaagcgacgccatcttcatcttttacgcgattagcctcatggctatttgtgccgaagtgggagttgtatggtagcagtgaggagattgtggctacgacacaggcgggttctcttgagcggcttacatctccgcattaggcctgcgtacgatccagatcatgggaaactttacaatggcttactcgttttatctcaacactgagcttccaattcactctatgcattgattaacacgtttggtcatgtggttcttcagctgtaaatcttcagcttcccaagaattgcaacctcgctgattgctaatagtgttgcatgcgttgcatcctggtgcggcagtgcaaaggagagtcaaagtagccggcagattaatttaagcttatatcactcaggggtaaacagccgtaaaggaccttttgatctaacatgccgatgtgtatgtagatcacgcaatgcccaccatatcttggcagtcagatttgtccgtggctccgtctcctcgtgatactgcaaagcacatatggcgtacagctgtgatcaagagtccgtctgggaggtctcttgtatatgtactgcttggtttacatttgtatacagatgcgcatcctatggctgttattgatctcgacctcttccatcaattgtcccaatagttctgcaaagagggcttggacaactgaagagacacccaaattggattcagcgaaggaaacccaacagcagattgttctgtatcgtattgctcttacatacatttcagcctaatactcttgtcccagcaagtggccattcgaaacgcccaaccaaggggacaattggctgctccgatgaagatattagcccctgctatatcgcattaggctgtcggggtggtctggatgaaacgtcttggccaaatcgtgatcgattgatactcgcatctataagatggcacagatcgactcttgattcacagacatccgtcagccctcaagccgtttgcaagtccacaaacacaagcacaagcatagcgtcgcaatgaagttccttcaagtcctccctgccctcataccggccgccctggcccaaaccagctgtgaccagtgggcaaccttcactggcaacggctacacagtcagcaacaacctttggggagcatcagccggctctggatttggctgcgtgacggcggtatcgctcagcggcggggcctcctggcacgcagactggcagtggtccggcggccagaacaacgtcaagtcgtaccagaactctcagattgccattccccagaagaggaccgtcaacagcatcagcagcatgcccaccactgccagctggagctacagcgggagcaacatccgcgctaatgttgcgtatgacttgttcaccgcagccaacccgaatcatgtcacgtactcgggagactacgaactcatgatctggtaagccataagaagtgaccctccttgatagtttcgactaacaacatgtcttgaggcttggcaaatacggcgatattgggccgattgggtcctcacagggaacagtcaacgtcggtggccagagctggacgctctactatggctacaacggagccatgcaagtctattcctttgtggcccagaccaacactaccaactacagcggagatgtcaagaacttcttcaattatctccgagacaataaaggatacaacgctgcaggccaatatgttcttagtaagtcaccctcactgtgactgggctgagtttgttgcaacgtttgctaacaaaaccttcgtataggctaccaatttggtaccgagcccttcacgggcagtggaactctgaacgtcgcatcctggaccgcatctatcaactaaaacctggaaacgtgagatgtggtgggcatacgttattgagcgagggaaaaaaagcattggatccattgaagatgttagtcatatacagacttagaagatttacatgaatgtcaaacgatgagcgactgtggaacgttatgaataatagactggaaccgggccctttgattgacgactccatattttgtagatgtagcaactcggcaagagcattatgtgcaatacatttgttaccatacaaaggcagctgccagacgacttgtattgcgtacaattctcacggcaagctttccaggtgttatgcattatgcgcaaatgcttgatgcttaccgcaggattaatctcggaagaagcgctgcaagctatatgggtgtagtagatatgtagatgtaccaaccaatgaagaacatttatggtctagaacgtagtgatgaaggttttgagtaatttgtatcaagtaagacgatattattgatataataccaagcatatattcatgataaattacttggaaccacccttgcgtccggcctcacgagccttctcactgccgggctcgaaggagccactggaggcctgtccacccttggatgcgatttcctgcaccttttccttgggcctgcacgtcgattagacatgattcaaatcgagatcttggaatatcttacatgctggcgaagccaccggtgtggctggactgtccgcccttctgcgcaatgctttgaacctcctccttggggctgtgtagaaaggtttgttagcaacattactacaactctcaggactcggtggtcgtaccggttggcgaagtttccggggttatcgttgccagacattgtgtgattatttggtgtgcaaatgtgtgctatgtgtgttgttgctgttggtgatgatgctgaagctgttgaaagcaggctggttctgtgggagagacttgggat

SEQ ID NO: 48 - DNA, 35 bp, synthetic construct
  source 1..35: mol_type = other DNA
agagaggccgaagctgcccagaaccagacggagac

SEQ ID NO: 49 - DNA, 35 bp, synthetic construct
  source 1..35: mol_type = other DNA
gcggccgcccctttatcaagcaaacttcaacctct